European Patent Application EP 4 385 524 A1, published June 19, 2024. Title: MSH2 또는 MSH6 억제제를 유효성분으로 포함하는 암 예방 또는 치료용 조성물. Applicant: 주식회사 네오나. Application WO. The sequence listing filed with the application follows.

SEQUENCE LISTING (2 sequences)

SEQ ID NO: 1 - RNA, 21 nt, synthetic construct
  source 1..21: mol_type = other RNA
tctgcagagtgttgtgctttt

SEQ ID NO: 2 - RNA, 21 nt, synthetic construct
  source 1..21: mol_type = other RNA
gccagacactaaggaggaatt